European Patent Application EP 4 800 111 A1, published September 2, 2026. Title: 一种抵抗狂犬病毒的mRNA疫苗及其制备方法. Applicant: 石药集团巨石生物制药有限公司. The sequence listing filed with the application follows.

SEQUENCE LISTING (10 sequences)

SEQ ID NO: 1 - RNA, 2113 nt, synthetic construct
  source 1..2113: mol_type = other RNA
gggagacccaagctggctagcgtttaaacttaagcttggtaccgagctcggatccactagtccagtgtggtggaattcagaataaactagtattcttctggtccccacagactcagagagaacccgccaccatgatccctcaggccctgctgttcgtgcccctgctggtgtttcctctgtgcttcggcaagttcccaatctacaccatcccagataagctgggaccttggagccctatcgacattcaccacctgagttgtcctaacaacctggtggtcgaggacgagggctgtaccaatctgagcggcttctcctacatggaactgaaggtgggctacatcagcgccatcaaggtgaacggcttcacttgcaccggcgtggtgaccgaggccgagacatacacaaatttcgttggctacgtgaccaccaccttcaagagaaagcacttccgccccacccctgacgcctgtcggagcgcttacaactggaagatggccggcgatcctagatacgaggaaagtctgcacaacccctatcctgattaccactggctgagaaccgtgaagaccacaaaggaaagcgtggtgatcattagccctagcgtggccgatctggacccttacgacaagtctctccatagcagagtgttccctagaggcaagtgcagcggcataacagtgagctccgcctactgcagcaccaatcacgactacaccatctggatgcctgagaaccctagactgggtacatcttgtgatatcttcacaaacagcagaggcaaacgggcttctaaaggcagcaagacctgtggctttgtggacgagcggggactgtacaaatctctgaagggcgcctgcaagctgaaactgtgcggcgtgctgggcctccggctgatggacggcacctgggtcgccatccagaccagcaacgagacaaagtggtgcccccccgatcagctggtgaatctgcacgatttccacagcgacgaaatcgagcatctggtggtggaagaactggttaaaaagcgggaagagtgcctggatgctctggaaagcatcatgacaaccaaatccgtgagcttccggaggctgagccacctgagaaagctggttcccggcttcggcaaggcctataccatctttaacaagacactgatggaagccgacgcccactacaagagcgtccggacctggaacgagatcatccctagcaagggctgcctgagagtgggcggaagatgccacccccacgtgaacggcgtgtttttcaacggcatcatcctgggccctgacggccacgtgctgatccctgagatgcagtccagcctgctgcagcagcacatggaactgctggagagctctgtgatccccctgatgcaccctctggccgaccccagcacagtgtttaaggacggcgacgaggtggaggacttcgtggaagtgcacctgcctgacgtgcataagcaggtgagcggcgtggacctgggactgccaaactggggaaaagacgtgctgatgggcgctggcgtgctgaccgccctgatgctgatgatcttcctgatgacatgctgcagaagaaccaaccgggccgagagcatccaacacagcctgggcgagaccggcagaaaggtgtcggtcacctctcagtctggaagagtgatcagctcttgggagagctacaagagcggaggagaaaccaaactgtgataactcgagctggtactgcatgcacgcaatgctagctgcccctttcccgtcctgggtaccccgagtctcccccgacctcgggtcccaggtatgctcccacctccacctgccccactcaccacctctgctagttccagacacctcccaagcacgcagcaatgcagctcaaaacgcttagcctagccacacccccacgggaaacagcagtgattaacctttagcaataaacgaaagtttaactaagctatactaaccccagggttggtcaatttcgtgccagccacaccctggagctagcaaaaaaaaaaaaaaaaaaaaaaaaaaaaaagcatatgactaaaaaaaaaaaaaaaaaaaaaaaaaaaaaaaaaaaaaaaaaaaaaaaaaaaaaaaaaaaaaaaaaaaaa

SEQ ID NO: 2 - RNA, 2113 nt, synthetic construct
  source 1..2113: mol_type = other RNA
gggagacccaagctggctagcgtttaaacttaagcttggtaccgagctcggatccactagtccagtgtggtggaattcagaataaactagtattcttctggtccccacagactcagagagaacccgccaccatgattccccaggcactgctgttcgtgccgttgctggtttttccactgtgttttggtaagtttcccatatataccatccccgataaactgggcccttggtcccccatcgacatccaccacttgagctgtcccaacaatctggttgttgaggacgagggctgtaccaacctcagcggcttcagttatatggaactgaaggttggctatattagcgccatcaaagtgaatggctttacctgcaccggagtggtgaccgaagccgagacctacacgaactttgttggttacgtcaccacaacgtttaaacgtaagcacttccgaccgactccagatgcctgtaggtcggcctacaattggaagatggccggagatccacgttatgaggaatccctccataacccatacccggactaccattggctgaggacggtgaagacaacgaaggagtccgtggtcataatctcgccatccgtggccgacctggatccctacgataagagcctgcactcccgagtgttcccacgaggcaagtgtagcggtattacggtcagcagcgcatactgttccacaaatcacgattatactatatggatgcccgagaacccacggctgggaacaagttgcgacatttttaccaattccaggggaaagcgggcatcgaagggatccaagacatgtggcttcgtcgatgaacggggactgtacaagagtcttaaaggcgcttgtaagctgaaactctgtggtgttctgggattgcgactgatggatggaacctgggtggccattcagacgagcaatgagaccaaatggtgcccgcccgatcaattggtgaatctgcatgactttcacagcgacgagatcgagcatttggtggtggaggaactggtgaagaagcgcgaagagtgcttggacgccctggaatcgatcatgaccactaaatcggtttcgttccgccggctttcgcacctcaggaagttggtgccgggcttcggcaaggcttacaccatttttaataagaccctgatggaggctgacgcacactacaagtccgttaggacttggaatgagatcattccaagtaagggctgcttgagggtaggaggtcggtgccatccgcatgtgaatggtgtcttcttcaatggcatcattttgggaccggatggccatgtgctcatcccagagatgcagtcctccctcctccaacagcacatggaactgctggagagttcggtaattccactgatgcatcccctggccgatccgagcacagtttttaaggacggtgatgaggtagaagacttcgtcgaggtacatttgcccgatgtacacaaacaggtttcgggagtggaccttggattgcccaactggggcaaggatgttttgatgggagccggagtgctcaccgcacttatgctgatgattttcctgatgacttgctgccgcaggaccaacagggcagagtcgattcagcatagcttgggcgagacgggtcggaaagtctccgtcaccagtcagtccggacgtgtgatcagctcctgggagagttacaaaagcggcggtgaaaccaagctgtgataactcgagctggtactgcatgcacgcaatgctagctgcccctttcccgtcctgggtaccccgagtctcccccgacctcgggtcccaggtatgctcccacctccacctgccccactcaccacctctgctagttccagacacctcccaagcacgcagcaatgcagctcaaaacgcttagcctagccacacccccacgggaaacagcagtgattaacctttagcaataaacgaaagtttaactaagctatactaaccccagggttggtcaatttcgtgccagccacaccctggagctagcaaaaaaaaaaaaaaaaaaaaaaaaaaaaaagcatatgactaaaaaaaaaaaaaaaaaaaaaaaaaaaaaaaaaaaaaaaaaaaaaaaaaaaaaaaaaaaaaaaaaaaaa

SEQ ID NO: 3 - RNA, 2115 nt, synthetic construct
  source 1..2115: mol_type = other RNA
gggagacccaagctggctagcgtttaaacttaagcttggtaccgagctcggatccactagtccagtgtggtggaattcagaataaactagtattcttctggtccccacagactcagagagaacccgccaccatgatcccccaagctttgctgttcgtgcctctcctggtctttccactgtgctttgggaaattccccatttacaccatcccagataagctcggcccttggtctcccatcgacattcatcacctgtcttgtcctaacaatttggtggtggaggacgaaggatgcacaaatcttagcggcttcagctatatggaattgaaagtcgggtacataagcgccattaaggtcaacggtttcacctgcacgggcgtggtgactgaggcggaaacttacacaaactttgtcggctatgtgaccacgacattcaagaggaaacacttcagacctacgccagatgcttgcaggtctgcttataactggaagatggcaggcgatcctaggtatgaggaatctctgcataacccttatcctgattatcattggcttcgcacggtgaaaaccaccaaagagagcgtggtcattatttcaccatctgtggcggatctggacccctacgacaaatctctgcactcaagagtgtttcctcggggcaaatgctcaggtatcaccgtttctagtgcctactgcagtacgaaccacgactacaccatttggatgcccgagaaccctaggttgggcacctcttgtgatatattcactaactctaggggaaagcgggcgtctaaagggtcaaagacctgcggattcgttgacgagaggggactgtataagagcttgaagggcgcctgcaagctgaaactgtgcggggtgcttggattgcgcctgatggatggcacctgggtggccattcagacaagcaatgaaaccaagtggtgtccgcccgatcagcttgtgaacctgcatgactttcattctgacgagatcgaacacctcgtggtcgaggagctggtgaaaaagagggaagaatgcctggatgcgctcgagagcattatgactaccaaaagcgtgagcttcaggcgattgagccacctgcgcaagttggtgcctggcttcgggaaggcttatactatttttaacaagactcttatggaggcagacgctcattacaagagcgtcaggacctggaatgaaattattcccagcaagggctgcctgagagttgggggacggtgtcaccctcacgttaacggcgtgttcttcaacggcatcatcctgggtcccgacggtcatgtgctgatccccgaaatgcaaagttctctgctccaacagcacatggaactgctggagtcctccgtgatcccactgatgcaccccctggctgacccctctacagtgttcaaagatggggacgaagtcgaagactttgtggaggtccacctgcccgacgtgcacaaacaggtctcaggagtggatttgggactcccaaattggggcaaagatgtcctgatgggtgcgggggtcctgacagctctgatgctcatgatattccttatgacatgttgcaggcgcaccaacagggccgagagtatccagcacagcttgggtgagactgggcggaaggtgtccgttacatcccagtctggcagggttatctcatcctgggagtcctacaagtctggaggcgagactaaactgtgataactcgagctggtactgcatgcacgcaatgctagctgcccctttcccgtcctgggtaccccgagtctcccccgacctcgggtcccaggtatgctcccacctccacctgccccactcaccacctctgctagttccagacacctcccaagcacgcagcaatgcagctcaaaacgcttagcctagccacacccccacgggaaacagcagtgattaacctttagcaataaacgaaagtttaactaagctatactaaccccagggttggtcaatttcgtgccagccacaccctggagctagcaaaaaaaaaaaaaaaaaaaaaaaaaaaaaagcatatgactaaaaaaaaaaaaaaaaaaaaaaaaaaaaaaaaaaaaaaaaaaaaaaaaaaaaaaaaaaaaaaaaaaaaaaa

SEQ ID NO: 4 - protein, 524 aa, Rabies virus
MIPQALLFVPLLVFPLCFGKFPIYTIPDKLGPWSPIDIHHLSCPNNLVVEDEGCTNLSGFSYMELKVGYISAIKVNGFTCTGVVTEAETYTNFVGYVTTTFKRKHFRPTPDACRSAYNWKMAGDPRYEESLHNPYPDYHWLRTVKTTKESVVIISPSVADLDPYDKSLHSRVFPRGKCSGITVSSAYCSTNHDYTIWMPENPRLGTSCDIFTNSRGKRASKGSKTCGFVDERGLYKSLKGACKLKLCGVLGLRLMDGTWVAIQTSNETKWCPPDQLVNLHDFHSDEIEHLVVEELVKKREECLDALESIMTTKSVSFRRLSHLRKLVPGFGKAYTIFNKTLMEADAHYKSVRTWNEIIPSKGCLRVGGRCHPHVNGVFFNGIILGPDGHVLIPEMQSSLLQQHMELLESSVIPLMHPLADPSTVFKDGDEVEDFVEVHLPDVHKQVSGVDLGLPNWGKDVLMGAGVLTALMLMIFLMTCCRRTNRAESIQHSLGETGRKVSVTSQSGRVISSWESYKSGGETKL

SEQ ID NO: 5 - skipped

SEQ ID NO: 6 - DNA, 131 bp, unidentified
  source 1..131: mol_type = other DNA
gggagacccaagctggctagcgtttaaacttaagcttggtaccgagctcggatccactagtccagtgtggtggaattcagaataaactagtattcttctggtccccacagactcagagagaacccgccacc

SEQ ID NO: 7 - DNA, 110 bp, unidentified
  source 1..110: mol_type = other DNA
aaaaaaaaaaaaaaaaaaaaaaaaaaaaaagcatatgactaaaaaaaaaaaaaaaaaaaaaaaaaaaaaaaaaaaaaaaaaaaaaaaaaaaaaaaaaaaaaaaaaaaaaa

SEQ ID NO: 8 - DNA, 142 bp, unidentified
  source 1..142: mol_type = other DNA
ctcgagctggtactgcatgcacgcaatgctagctgcccctttcccgtcctgggtaccccgagtctcccccgacctcgggtcccaggtatgctcccacctccacctgccccactcaccacctctgctagttccagacacctcc

SEQ ID NO: 9 - DNA, 139 bp, unidentified
  source 1..139: mol_type = other DNA
caagcacgcagcaatgcagctcaaaacgcttagcctagccacacccccacgggaaacagcagtgattaacctttagcaataaacgaaagtttaactaagctatactaaccccagggttggtcaatttcgtgccagccac

SEQ ID NO: 10 - DNA, 2113 bp, synthetic construct
  source 1..2113: mol_type = other DNA
gggagacccaagctggctagcgtttaaacttaagcttggtaccgagctcggatccactagtccagtgtggtggaattcagaataaactagtattcttctggtccccacagactcagagagaacccgccaccatgatccctcaggccctgctgttcgtgcccctgctggtgtttcctctgtgcttcggcaagttcccaatctacaccatcccagataagctgggaccttggagccctatcgacattcaccacctgagttgtcctaacaacctggtggtcgaggacgagggctgtaccaatctgagcggcttctcctacatggaactgaaggtgggctacatcagcgccatcaaggtgaacggcttcacttgcaccggcgtggtgaccgaggccgagacatacacaaatttcgttggctacgtgaccaccaccttcaagagaaagcacttccgccccacccctgacgcctgtcggagcgcttacaactggaagatggccggcgatcctagatacgaggaaagtctgcacaacccctatcctgattaccactggctgagaaccgtgaagaccacaaaggaaagcgtggtgatcattagccctagcgtggccgatctggacccttacgacaagtctctccatagcagagtgttccctagaggcaagtgcagcggcataacagtgagctccgcctactgcagcaccaatcacgactacaccatctggatgcctgagaaccctagactgggtacatcttgtgatatcttcacaaacagcagaggcaaacgggcttctaaaggcagcaagacctgtggctttgtggacgagcggggactgtacaaatctctgaagggcgcctgcaagctgaaactgtgcggcgtgctgggcctccggctgatggacggcacctgggtcgccatccagaccagcaacgagacaaagtggtgcccccccgatcagctggtgaatctgcacgatttccacagcgacgaaatcgagcatctggtggtggaagaactggttaaaaagcgggaagagtgcctggatgctctggaaagcatcatgacaaccaaatccgtgagcttccggaggctgagccacctgagaaagctggttcccggcttcggcaaggcctataccatctttaacaagacactgatggaagccgacgcccactacaagagcgtccggacctggaacgagatcatccctagcaagggctgcctgagagtgggcggaagatgccacccccacgtgaacggcgtgtttttcaacggcatcatcctgggccctgacggccacgtgctgatccctgagatgcagtccagcctgctgcagcagcacatggaactgctggagagctctgtgatccccctgatgcaccctctggccgaccccagcacagtgtttaaggacggcgacgaggtggaggacttcgtggaagtgcacctgcctgacgtgcataagcaggtgagcggcgtggacctgggactgccaaactggggaaaagacgtgctgatgggcgctggcgtgctgaccgccctgatgctgatgatcttcctgatgacatgctgcagaagaaccaaccgggccgagagcatccaacacagcctgggcgagaccggcagaaaggtgtcggtcacctctcagtctggaagagtgatcagctcttgggagagctacaagagcggaggagaaaccaaactgtgataactcgagctggtactgcatgcacgcaatgctagctgcccctttcccgtcctgggtaccccgagtctcccccgacctcgggtcccaggtatgctcccacctccacctgccccactcaccacctctgctagttccagacacctcccaagcacgcagcaatgcagctcaaaacgcttagcctagccacacccccacgggaaacagcagtgattaacctttagcaataaacgaaagtttaactaagctatactaaccccagggttggtcaatttcgtgccagccacaccctggagctagcaaaaaaaaaaaaaaaaaaaaaaaaaaaaaagcatatgactaaaaaaaaaaaaaaaaaaaaaaaaaaaaaaaaaaaaaaaaaaaaaaaaaaaaaaaaaaaaaaaaaaaaa